European Patent Application EP 4 163 295 A1, published April 12, 2023. Title: WNT SIGNALING AGONIST MOLECULES. Applicant: Universite Libre de Bruxelles. The sequence listing filed with the application follows.

SEQUENCE LISTING (121 sequences)

SEQ ID NO: 1 - protein, 1338 aa, Homo sapiens
  SOURCE 1..1338
MGAGGRRMRGAPARLLLPLLPWLLLLLAPEARGAPGCPLSIRSCKCSGERPKGLSGGVPGPARRRVVCSGGDLPEPPEPGLLPNGTVTLLLSNNKITGLRNGSFLGLSLLEKLDLRNNIISTVQPGAFLGLGELKRLDLSNNRIGCLTSETFQGLPRLLRLNISGNIFSSLQPGVFDELPALKVVDLGTEFLTCDCHLRWLLPWAQNRSLQLSEHTLCAYPSALHAQALGSLQEAQLCCEGALELHTHHLIPSLRQVVFQGDRLPFQCSASYLGNDTRIRWYHNRAPVEGDEQAGILLAESLIHDCTFITSELTLSHIGVWASGEWECTVSMAQGNASKKVEIVVLETSASYCPAERVANNRGDFRWPRTLAGITAYQSCLQYPFTSVPLGGGAPGTRASRRCDRAGRWEPGDYSHCLYTNDITRVLYTFVLMPINASNALTLAHQLRVYTAEAASFSDMMDVVYVAQMIQKFLGYVDQIKELVEVMVDMASNLMLVDEHLLWLAQREDKACSRIVGALERIGGAALSPHAQHISVNARNVALEAYLIKPHSYVGLTCTAFQRREGGVPGTRPGSPGQNPPPEPEPPADQQLRFRCTTGRPNVSLSSFHIKNSVALASIQLPPSLFSSLPAALAPPVPPDCTLQLLVFRNGRLFHSHSNTSRPGAAGPGKRRGVATPVIFAGTSGCGVGNLTEPVAVSLRHWAEGAEPVAAWWSQEGPGEAGGWTSEGCQLRSSQPNVSALHCQHLGNVAVLMELSAFPREVGGAGAGLHPVVYPCTALLLLCLFATIITYILNHSSIRVSRKGWHMLLNLCFHIAMTSAVFAGGITLTNYQMVCQAVGITLHYSSLSTLLWMGVKARVLHKELTWRAPPPQEGDPALPTPSPMLRFYLIAGGIPLIICGITAAVNIHNYRDHSPYCWLVWRPSLGAFYIPVALILLITWIYFLCAGLRLRGPLAQNPKAGNSRASLEAGEELRGSTRLRGSGPLLSDSGSLLATGSARVGTPGPPEDGDSLYSPGVQLGALVTTHFLYLAMWACGALAVSQRWLPRVVCSCLYGVAASALGLFVFTHHCARRRDVRASWRACCPPASPAAPHAPPRALPAAAEDGSPVFGEGPPSLKSSPSGSSGHPLALGPCKLTNLQLAQSQVCEAGAAAGGEGEPEPAGTRGNLAHRHPNNVHHGRRAHKSRAKGHRAGEACGKNRLKALRGGAAGALELLSSESGSLHNSPTDSYLGSSRNSPGAGLQLEGEPMLTPSEGSDTSAAPLSEAGRAGQRRSASRDSLKGGGALEKESHRRSYPLNAASLNGAPKGGKYDDVTLMGAEVASGGCMKTGLWKSETTV

SEQ ID NO: 2 - protein, 971 aa, Homo sapiens
  SOURCE 1..971
MATVRASLRGALLLLLAVAGVAEVAGGLAPGSAGALCCNHSKDNQMCRDVCEQIFSSKSESRLKHLLQRAPDYCPETMVEIWNCMNSSLPGVFKKSDGWVGLGCCELAIALECRQACKQASSKNDISKVCRKEYENALFSCISRNEMGSVCCSYAGHHTNCREYCQAIFRTDSSPGPSQIKAVENYCASISPQLIHCVNNYTQSYPMRNPTDSLYCCDRAEDHACQNACKRILMSKKTEMEIVDGLIEGCKTQPLPQDPLWQCFLESSQSVHPGVTVHPPPSTGLDGAKLHCCSKANTSTCRELCTKLYSMSWGNTQSWQEFDRFCEYNPVEVSMLTCLADVREPCQLGCRNLTYCTNFNNRPTELFRSCNAQSDQGAMNDMKLWEKGSIKMPFINIPVLDIKKCQPEMWKAIACSLQIKPCHSKSRGSIICKSDCVEILKKCGDQNKFPEDHTAESICELLSPTDDLKNCIPLDTYLRPSTLGNIVEEVTHPCNPNPCPANELCEVNRKGCPSGDPCLPYFCVQGCKLGEASDFIVRQGTLIQVPSSAGEVGCYKICSCGQSGLLENCMEMHCIDLQKSCIVGGKRKSHGTSFSIDCNVCSCFAGNLVCSTRLCLSEHSSEDDRRTFTGLPCNCADQFVPVCGQNGRTYPSACIARCVGLQDHQFEFGSCMSKDPCNPNPCQKNQRCIPKPQVCLTTFDKFGCSQYECVPRQLACDQVQDPVCDTDHMEHNNLCTLYQRGKSLSYKGPCQPFCRATEPVCGHNGETYSSVCAAYSDRVAVDYYGDCQAVGVLSEHSSVAECASVKCPSLLAAGCKPIIPPGACCPLCAGMLRVLFDKEKLDTIAKVTNKKPITVLEILQKIRMHVSVPQCDVFGYFSIESEIVILIIPVDHYPKALQIEACNKEAEKIESLINSDSPTLASHVPLSALIISQVQVSSSVPSAGVRARPSCHSLLLPLSLGLALHLLWTYN

SEQ ID NO: 3 - protein, 1615 aa, Homo sapiens
  SOURCE 1..1615
MEAAPPGPPWPLLLLLLLLLALCGCPAPAAASPLLLFANRRDVRLVDAGGVKLESTIVVSGLEDAAAVDFQFSKGAVYWTDVSEEAIKQTYLNQTGAAVQNVVISGLVSPDGLACDWVGKKLYWTDSETNRIEVANLNGTSRKVLFWQDLDQPRAIALDPAHGYMYWTDWGETPRIERAGMDGSTRKIIVDSDIYWPNGLTIDLEEQKLYWADAKLSFIHRANLDGSFRQKVVEGSLTHPFALTLSGDTLYWTDWQTRSIHACNKRTGGKRKEILSALYSPMDIQVLSQERQPFFHTRCEEDNGGCSHLCLLSPSEPFYTCACPTGVQLQDNGRTCKAGAEEVLLLARRTDLRRISLDTPDFTDIVLQVDDIRHAIAIDYDPLEGYVYWTDDEVRAIRRAYLDGSGAQTLVNTEINDPDGIAVDWVARNLYWTDTGTDRIEVTRLNGTSRKILVSEDLDEPRAIALHPVMGLMYWTDWGENPKIECANLDGQERRVLVNASLGWPNGLALDLQEGKLYWGDAKTDKIEVINVDGTKRRTLLEDKLPHIFGFTLLGDFIYWTDWQRRSIERVHKVKASRDVIIDQLPDLMGLKAVNVAKVVGTNPCADRNGGCSHLCFFTPHATRCGCPIGLELLSDMKTCIVPEAFLVFTSRAAIHRISLETNNNDVAIPLTGVKEASALDFDVSNNHIYWTDVSLKTISRAFMNGSSVEHVVEFGLDYPEGMAVDWMGKNLYWADTGTNRIEVARLDGQFRQVLVWRDLDNPRSLALDPTKGYIYWTEWGGKPRIVRAFMDGTNCMTLVDKVGRANDLTIDYADQRLYWTDLDTNMIESSNMLGQERVVIADDLPHPFGLTQYSDYIYWTDWNLHSIERADKTSGRNRTLIQGHLDFVMDILVFHSSRQDGLNDCMHNNGQCGQLCLAIPGGHRCGCASHYTLDPSSRNCSPPTTFLLFSQKSAISRMIPDDQHSPDLILPLHGLRNVKAIDYDPLDKFIYWVDGRQNIKRAKDDGTQPFVLTSLSQGQNPDRQPHDLSIDIYSRTLFWTCEATNTINVHRLSGEAMGVVLRGDRDKPRAIVVNAERGYLYFTNMQDRAAKIERAALDGTEREVLFTTGLIRPVALVVDNTLGKLFWVDADLKRIESCDLSGANRLTLEDANIVQPLGLTILGKHLYWIDRQQQMIERVEKTTGDKRTRIQGRVAHLTGIHAVEEVSLEEFSAHPCARDNGGCSHICIAKGDGTPRCSCPVHLVLLQNLLTCGEPPTCSPDQFACATGEIDCIPGAWRCDGFPECDDQSDEEGCPVCSAAQFPCARGQCVDLRLRCDGEADCQDRSDEADCDAICLPNQFRCASGQCVLIKQQCDSFPDCIDGSDELMCEITKPPSDDSPAHSSAIGPVIGIILSLFVMGGVYFVCQRVVCQRYAGANGPFPHEYVSGTPHVPLNFIAPGGSQHGPFTGIACGKSMMSSVSLMGGRGGVPLYDRNHVTGASSSSSSSTKATLYPPILNPPPSPATDPSLYNMDMFYSSNIPATARPYRPYIIRGMAPPTTPCSTDVCDSDYSASRWKASKYYLDLNSDSDPYPPPPTPHSQYLSAEDSCPPSPATERSYFHLFPPPPSPCTDSS

SEQ ID NO: 4 - protein, 1613 aa, Homo sapiens
  SOURCE 1..1613
MGAVLRSLLACSFCVLLRAAPLLLYANRRDLRLVDATNGKENATIVVGGLEDAAAVDFVFSHGLIYWSDVSEEAIKRTEFNKTESVQNVVVSGLLSPDGLACDWLGEKLYWTDSETNRIEVSNLDGSLRKVLFWQELDQPRAIALDPSSGFMYWTDWGEVPKIERAGMDGSSRFIIINSEIYWPNGLTLDYEEQKLYWADAKLNFIHKSNLDGTNRQAVVKGSLPHPFALTLFEDILYWTDWSTHSILACNKYTGEGLREIHSDIFSPMDIHAFSQQRQPNATNPCGIDNGGCSHLCLMSPVKPFYQCACPTGVKLLENGKTCKDGATELLLLARRTDLRRISLDTPDFTDIVLQLEDIRHAIAIDYDPVEGYIYWTDDEVRAIRRSFIDGSGSQFVVTAQIAHPDGIAVDWVARNLYWTDTGTDRIEVTRLNGTMRKILISEDLEEPRAIVLDPMVGYMYWTDWGEIPKIERAALDGSDRVVLVNTSLGWPNGLALDYDEGKIYWGDAKTDKIEVMNTDGTGRRVLVEDKIPHIFGFTLLGDYVYWTDWQRRSIERVHKRSAEREVIIDQLPDLMGLKATNVHRVIGSNPCAEENGGCSHLCLYRPQGLRCACPIGFELISDMKTCIVPEAFLLFSRRADIRRISLETNNNNVAIPLTGVKEASALDFDVTDNRIYWTDISLKTISRAFMNGSALEHVVEFGLDYPEGMAVDWLGKNLYWADTGTNRIEVSKLDGQHRQVLVWKDLDSPRALALDPAEGFMYWTEWGGKPKIDRAAMDGSERTTLVPNVGRANGLTIDYAKRRLYWTDLDTNLIESSNMLGLNREVIADDLPHPFGLTQYQDYIYWTDWSRRSIERANKTSGQNRTIIQGHLDYVMDILVFHSSRQSGWNECASSNGHCSHLCLAVPVGGFVCGCPAHYSLNADNRTCSAPTTFLLFSQKSAINRMVIDEQQSPDIILPIHSLRNVRAIDYDPLDKQLYWIDSRQNMIRKAQEDGSQGFTVVVSSVPSQNLEIQPYDLSIDIYSRYIYWTCEATNVINVTRLDGRSVGVVLKGEQDRPRAVVVNPEKGYMYFTNLQERSPKIERAALDGTEREVLFFSGLSKPIALALDSRLGKLFWADSDLRRIESSDLSGANRIVLEDSNILQPVGLTVFENWLYWIDKQQQMIEKIDMTGREGRTKVQARIAQLSDIHAVKELNLQEYRQHPCAQDNGGCSHICLVKGDGTTRCSCPMHLVLLQDELSCGEPPTCSPQQFTCFTGEIDCIPVAWRCDGFTECEDHSDELNCPVCSESQFQCASGQCIDGALRCNGDANCQDKSDEKNCEVLCLIDQFRCANGQCIGKHKKCDHNVDCSDKSDELDCYPTEEPAPQATNTVGSVIGVIVTIFVSGTVYFICQRMLCPRMKGDGETMTNDYVVHGPASVPLGYVPHPSSLSGSLPGMSRGKSMISSLSIMGGSSGPPYDRAHVTGASSSSSSSTKGTYFPAILNPPPSPATERSHYTMEFGYSSNSPSTHRSYSYRPYSYRHFAPPTTPCSTDVCDSDYAPSRRMTSVATAKGYTSDLNYDSEPVPPPPTPRSQYLSAEENYESCPPSPYTERSYSHHLYPPPPSPCTDSS

SEQ ID NO: 5 - protein, 48 aa, Homo sapiens
  SOURCE 1..48
CCDRAEDHACQNACKRILMSKKTEMEIVDGLIEGCKTQPLPQDPLWQC

SEQ ID NO: 6 - protein, 47 aa, Homo sapiens
  SOURCE 1..47
CCSKANTSTCRELCTKLYSMSWGNTQSWQEFDRFCEYNPVEVSMLTC

SEQ ID NO: 7 - skipped

SEQ ID NO: 8 - protein, 4 aa, synthetic construct
  SOURCE 1..4
  REGION 1..4: NOTE = LRP repeat domain
YWTD

SEQ ID NO: 9 - skipped

SEQ ID NO: 10 - protein, 5 aa, synthetic construct
  SOURCE 1..5
  REGION 1..5: NOTE = LRP motif
PPPSP

SEQ ID NO: 11 - protein, 16 aa, synthetic construct
  SOURCE 1..16
  REGION 1..16: NOTE = Frizzled-binding domain
  SITE 1: NOTE = any amino acid
  SITE 3..6: NOTE = any amino acid
  SITE 9..15: NOTE = any amino acid
XKXXXXSGXXXXXXXW

SEQ ID NO: 12 - protein, 16 aa, Homo sapiens
  SOURCE 1..16
CKCHGVSGSCTTKTCW

SEQ ID NO: 13 - skipped

SEQ ID NO: 14 - protein, 89 aa, Homo sapiens
  SOURCE 1..89
MYHTKGQEGSVCLRSSDCASGLCCARHFWSKICKPVLKEGQVCTKHRRKGSHGLEIFQRCYCGEGLSCRIQKDHHQASNSSRLHTCQRH

SEQ ID NO: 15 - protein, 349 aa, Homo sapiens
  SOURCE 1..349
MNRKARRCLGHLFLSLGMVYLRIGGFSSVVALGASIICNKIPGLAPRQRAICQSRPDAIIVIGEGSQMGLDECQFQFRNGRWNCSALGERTVFGKELKVGSREAAFTYAIIAAGVAHAITAACTQGNLSDCGCDKEKQGQYHRDEGWKWGGCSADIRYGIGFAKVFVDAREIKQNARTLMNLHNNEAGRKILEENMKLECKCHGVSGSCTTKTCWTTLPQFRELGYVLKDKYNEAVHVEPVRASRNKRPTFLKIKKPLSYRKPMDTDLVYIEKSPNYCEEDPVTGSVGTQGRACNKTAPQASGCDLMCCGRGYNTHQYARVWQCNCKFHWCCYVKCNTCSERTEMYTCK

SEQ ID NO: 16 - protein, 349 aa, Homo sapiens
  SOURCE 1..349
MHRNFRKWIFYVFLCFGVLYVKLGALSSVVALGANIICNKIPGLAPRQRAICQSRPDAIIVIGEGAQMGINECQYQFRFGRWNCSALGEKTVFGQELRVGSREAAFTYAITAAGVAHAVTAACSQGNLSNCGCDREKQGYYNQAEGWKWGGCSADVRYGIDFSRRFVDAREIKKNARRLMNLHNNEAGRKVLEDRMQLECKCHGVSGSCTTKTCWTTLPKFREVGHLLKEKYNAAVQVEVVRASRLRQPTFLRIKQLRSYQKPMETDLVYIEKSPNYCEEDAATGSVGTQGRLCNRTSPGADGCDTMCCGRGYNTHQYTKVWQCNCKFHWCCFVKCNTCSERTEVFTCK

SEQ ID NO: 17 - protein, 42 aa, Homo sapiens
  SOURCE 1..42
HVEPVRASRNKRPTFLKIKKPLSYRKPMDTDLVYIEKSPNYC

SEQ ID NO: 18 - protein, 29 aa, Homo sapiens
  SOURCE 1..29
VEPVRASRNKRPTFLKIKKPLSYRKPMDT

SEQ ID NO: 19 - protein, 29 aa, Homo sapiens
  SOURCE 1..29
VEVVRASRLRQPTFLRIKQLRSYQKPMET

SEQ ID NO: 20 - protein, 29 aa, synthetic construct
  SOURCE 1..29
  REGION 1..29: NOTE = RECK-binding domain
  SITE 1..3: NOTE = any amino acid
  SITE 5: NOTE = any amino acid
  SITE 7: NOTE = any amino acid
  SITE 9..13: NOTE = any amino acid
  SITE 16: NOTE = any amino acid
  SITE 18..22: NOTE = any amino acid
  SITE 24: NOTE = any amino acid
  SITE 26..29: NOTE = any amino acid
XXXVXAXRXXXXXFLXIXXXXXYXKXXXX

SEQ ID NO: 21 - protein, 22 aa, synthetic construct
  SOURCE 1..22
  REGION 1..22: NOTE = RECK-binding domain
  SITE 2: NOTE = any amino acid
  SITE 4: NOTE = any amino acid
  SITE 6..10: NOTE = any amino acid
  SITE 13: NOTE = any amino acid
  SITE 15..19: NOTE = any amino acid
  SITE 21: NOTE = any amino acid
VXAXRXXXXXFLXIXXXXXYXK

SEQ ID NO: 22 - protein, 29 aa, synthetic construct
  SOURCE 1..29
  REGION 1..29: NOTE = RECK-binding domain
  SITE 1..3: NOTE = any amino acid
  SITE 5: NOTE = any amino acid
  SITE 7: NOTE = any amino acid
  SITE 9..13: NOTE = any amino acid
  SITE 16..24: NOTE = any amino acid
  SITE 26..29: NOTE = any amino acid
XXXVXAXRXXXXXFLXXXXXXXXXKXXXX

SEQ ID NO: 23 - protein, 22 aa, synthetic construct
  SOURCE 1..22
  REGION 1..22: NOTE = RECK-binding domain
  SITE 2: NOTE = any amino acid
  SITE 4: NOTE = any amino acid
  SITE 6..10: NOTE = any amino acid
  SITE 13..21: NOTE = any amino acid
VXAXRXXXXXFLXXXXXXXXXK

SEQ ID NO: 24 - protein, 247 aa, synthetic construct
  SOURCE 1..247
  REGION 1..247: NOTE = N-terminal domain (NTD) of human Wnt7a polypeptide
LGASIICNKIPGLAPRQRAICQSRPDAIIVIGEGSQMGLDECQFQFRNGRWNCSALGERTVFGKELKVGSREAAFTYAIIAAGVAHAITAACTQGNLSDCGCDKEKQGQYHRDEGWKWGGCSADIRYGIGFAKVFVDAREIKQNARTLMNLHNNEAGRKILEENMKLECKCHGVSGSCTTKTCWTTLPQFRELGYVLKDKYNEAVHVEPVRASRNKRPTFLKIKKPLSYRKPMDTDLVYIEKSPNYC

SEQ ID NO: 25 - protein, 247 aa, synthetic construct
  SOURCE 1..247
  REGION 1..247: NOTE = N-terminal domain (NTD) of human Wnt7b polypeptide
LGANIICNKIPGLAPRQRAICQSRPDAIIVIGEGAQMGINECQYQFRFGRWNCSALGEKTVFGQELRVGSREAAFTYAITAAGVAHAVTAACSQGNLSNCGCDREKQGYYNQAEGWKWGGCSADVRYGIDFSRRFVDAREIKKNARRLMNLHNNEAGRKVLEDRMQLECKCHGVSGSCTTKTCWTTLPKFREVGHLLKEKYNAAVQVEVVRASRLRQPTFLRIKQLRSYQKPMETDLVYIEKSPNYC

SEQ ID NO: 26 - protein, 31 aa, synthetic construct
  SOURCE 1..31
  REGION 1..31: NOTE = signal peptide human Wnt7a polypeptide
MNRKARRCLGHLFLSLGMVYLRIGGFSSVVA

SEQ ID NO: 27 - protein, 31 aa, synthetic construct
  SOURCE 1..31
  REGION 1..31: NOTE = signal peptide human Wnt7b polypeptide
MHRNFRKWIFYVFLCFGVLYVKLGALSSVVA

SEQ ID NO: 28 - protein, 247 aa, synthetic construct
  SOURCE 1..247
  REGION 1..247: NOTE = human N-terminal domain (NTD) Wnt7a variant K159A
LGASIICNKIPGLAPRQRAICQSRPDAIIVIGEGSQMGLDECQFQFRNGRWNCSALGERTVFGKELKVGSREAAFTYAIIAAGVAHAITAACTQGNLSDCGCDKEKQGQYHRDEGWKWGGCSADIRYGIGFAKVFVDAREIKQNARTLMNLHNNEAGRAILEENMKLECKCHGVSGSCTTKTCWTTLPQFRELGYVLKDKYNEAVHVEPVRASRNKRPTFLKIKKPLSYRKPMDTDLVYIEKSPNYC

SEQ ID NO: 29 - protein, 247 aa, synthetic construct
  SOURCE 1..247
  REGION 1..247: NOTE = human N-terminal domain (NTD) Wnt7a variant A27R
LGASIICNKIPGLAPRQRAICQSRPDRIIVIGEGSQMGLDECQFQFRNGRWNCSALGERTVFGKELKVGSREAAFTYAIIAAGVAHAITAACTQGNLSDCGCDKEKQGQYHRDEGWKWGGCSADIRYGIGFAKVFVDAREIKQNARTLMNLHNNEAGRKILEENMKLECKCHGVSGSCTTKTCWTTLPQFRELGYVLKDKYNEAVHVEPVRASRNKRPTFLKIKKPLSYRKPMDTDLVYIEKSPNYC

SEQ ID NO: 30 - protein, 247 aa, synthetic construct
  SOURCE 1..247
  REGION 1..247: NOTE = human N-terminal domain (NTD) Wnt7a variant E33A
LGASIICNKIPGLAPRQRAICQSRPDAIIVIGAGSQMGLDECQFQFRNGRWNCSALGERTVFGKELKVGSREAAFTYAIIAAGVAHAITAACTQGNLSDCGCDKEKQGQYHRDEGWKWGGCSADIRYGIGFAKVFVDAREIKQNARTLMNLHNNEAGRKILEENMKLECKCHGVSGSCTTKTCWTTLPQFRELGYVLKDKYNEAVHVEPVRASRNKRPTFLKIKKPLSYRKPMDTDLVYIEKSPNYC

SEQ ID NO: 31 - protein, 247 aa, synthetic construct
  SOURCE 1..247
  REGION 1..247: NOTE = human N-terminal domain (NTD)Wnt7a variant E41A
LGASIICNKIPGLAPRQRAICQSRPDAIIVIGEGSQMGLDACQFQFRNGRWNCSALGERTVFGKELKVGSREAAFTYAIIAAGVAHAITAACTQGNLSDCGCDKEKQGQYHRDEGWKWGGCSADIRYGIGFAKVFVDAREIKQNARTLMNLHNNEAGRKILEENMKLECKCHGVSGSCTTKTCWTTLPQFRELGYVLKDKYNEAVHVEPVRASRNKRPTFLKIKKPLSYRKPMDTDLVYIEKSPNYC

SEQ ID NO: 32 - protein, 247 aa, synthetic construct
  SOURCE 1..247
  REGION 1..247: NOTE = human N-terminal domain (NTD)Wnt7a variant F44A
LGASIICNKIPGLAPRQRAICQSRPDAIIVIGEGSQMGLDECQAQFRNGRWNCSALGERTVFGKELKVGSREAAFTYAIIAAGVAHAITAACTQGNLSDCGCDKEKQGQYHRDEGWKWGGCSADIRYGIGFAKVFVDAREIKQNARTLMNLHNNEAGRKILEENMKLECKCHGVSGSCTTKTCWTTLPQFRELGYVLKDKYNEAVHVEPVRASRNKRPTFLKIKKPLSYRKPMDTDLVYIEKSPNYC

SEQ ID NO: 33 - protein, 247 aa, synthetic construct
  SOURCE 1..247
  REGION 1..247: NOTE = human N-terminal domain (NTD)Wnt7a variant N52Q
LGASIICNKIPGLAPRQRAICQSRPDAIIVIGEGSQMGLDECQFQFRNGRWQCSALGERTVFGKELKVGSREAAFTYAIIAAGVAHAITAACTQGNLSDCGCDKEKQGQYHRDEGWKWGGCSADIRYGIGFAKVFVDAREIKQNARTLMNLHNNEAGRKILEENMKLECKCHGVSGSCTTKTCWTTLPQFRELGYVLKDKYNEAVHVEPVRASRNKRPTFLKIKKPLSYRKPMDTDLVYIEKSPNYC

SEQ ID NO: 34 - protein, 247 aa, synthetic construct
  SOURCE 1..247
  REGION 1..247: NOTE = human N-terminal domain (NTD)Wnt7a variant I129A
LGASIICNKIPGLAPRQRAICQSRPDAIIVIGEGSQMGLDECQFQFRNGRWNCSALGERTVFGKELKVGSREAAFTYAIIAAGVAHAITAACTQGNLSDCGCDKEKQGQYHRDEGWKWGGCSADIRYGAGFAKVFVDAREIKQNARTLMNLHNNEAGRKILEENMKLECKCHGVSGSCTTKTCWTTLPQFRELGYVLKDKYNEAVHVEPVRASRNKRPTFLKIKKPLSYRKPMDTDLVYIEKSPNYC

SEQ ID NO: 35 - protein, 247 aa, synthetic construct
  SOURCE 1..247
  REGION 1..247: NOTE = human N-terminal domain (NTD)Wnt7a variant F131A
LGASIICNKIPGLAPRQRAICQSRPDAIIVIGEGSQMGLDECQFQFRNGRWNCSALGERTVFGKELKVGSREAAFTYAIIAAGVAHAITAACTQGNLSDCGCDKEKQGQYHRDEGWKWGGCSADIRYGIGAAKVFVDAREIKQNARTLMNLHNNEAGRKILEENMKLECKCHGVSGSCTTKTCWTTLPQFRELGYVLKDKYNEAVHVEPVRASRNKRPTFLKIKKPLSYRKPMDTDLVYIEKSPNYC

SEQ ID NO: 36 - protein, 247 aa, synthetic construct
  SOURCE 1..247
  REGION 1..247: NOTE = human N-terminal domain (NTD) Wnt7a variant K133A
LGASIICNKIPGLAPRQRAICQSRPDAIIVIGEGSQMGLDECQFQFRNGRWNCSALGERTVFGKELKVGSREAAFTYAIIAAGVAHAITAACTQGNLSDCGCDKEKQGQYHRDEGWKWGGCSADIRYGIGFAAVFVDAREIKQNARTLMNLHNNEAGRKILEENMKLECKCHGVSGSCTTKTCWTTLPQFRELGYVLKDKYNEAVHVEPVRASRNKRPTFLKIKKPLSYRKPMDTDLVYIEKSPNYC

SEQ ID NO: 37 - protein, 247 aa, synthetic construct
  SOURCE 1..247
  REGION 1..247: NOTE = human N-terminal domain (NTD) Wnt7a variant I141A
LGASIICNKIPGLAPRQRAICQSRPDAIIVIGEGSQMGLDECQFQFRNGRWNCSALGERTVFGKELKVGSREAAFTYAIIAAGVAHAITAACTQGNLSDCGCDKEKQGQYHRDEGWKWGGCSADIRYGIGFAKVFVDAREAKQNARTLMNLHNNEAGRKILEENMKLECKCHGVSGSCTTKTCWTTLPQFRELGYVLKDKYNEAVHVEPVRASRNKRPTFLKIKKPLSYRKPMDTDLVYIEKSPNYC

SEQ ID NO: 38 - protein, 247 aa, synthetic construct
  SOURCE 1..247
  REGION 1..247: NOTE = human N-terminal domain (NTD) Wnt7a variant R158A
LGASIICNKIPGLAPRQRAICQSRPDAIIVIGEGSQMGLDECQFQFRNGRWNCSALGERTVFGKELKVGSREAAFTYAIIAAGVAHAITAACTQGNLSDCGCDKEKQGQYHRDEGWKWGGCSADIRYGIGFAKVFVDAREIKQNARTLMNLHNNEAGAKILEENMKLECKCHGVSGSCTTKTCWTTLPQFRELGYVLKDKYNEAVHVEPVRASRNKRPTFLKIKKPLSYRKPMDTDLVYIEKSPNYC

SEQ ID NO: 39 - protein, 247 aa, synthetic construct
  SOURCE 1..247
  REGION 1..247: NOTE = human N-terminal domain (NTD) Wnt7a variant K181A
LGASIICNKIPGLAPRQRAICQSRPDAIIVIGEGSQMGLDECQFQFRNGRWNCSALGERTVFGKELKVGSREAAFTYAIIAAGVAHAITAACTQGNLSDCGCDKEKQGQYHRDEGWKWGGCSADIRYGIGFAKVFVDAREIKQNARTLMNLHNNEAGRKILEENMKLECKCHGVSGSCTTATCWTTLPQFRELGYVLKDKYNEAVHVEPVRASRNKRPTFLKIKKPLSYRKPMDTDLVYIEKSPNYC

SEQ ID NO: 40 - protein, 247 aa, synthetic construct
  SOURCE 1..247
  REGION 1..247: NOTE = human N-terminal domain (NTD) Wnt7a variant R191A
LGASIICNKIPGLAPRQRAICQSRPDAIIVIGEGSQMGLDECQFQFRNGRWNCSALGERTVFGKELKVGSREAAFTYAIIAAGVAHAITAACTQGNLSDCGCDKEKQGQYHRDEGWKWGGCSADIRYGIGFAKVFVDAREIKQNARTLMNLHNNEAGRKILEENMKLECKCHGVSGSCTTKTCWTTLPQFAELGYVLKDKYNEAVHVEPVRASRNKRPTFLKIKKPLSYRKPMDTDLVYIEKSPNYC

SEQ ID NO: 41 - protein, 247 aa, synthetic construct
  SOURCE 1..247
  REGION 1..247: NOTE = human N-terminal domain (NTD) Wnt7a variant K198A
LGASIICNKIPGLAPRQRAICQSRPDAIIVIGEGSQMGLDECQFQFRNGRWNCSALGERTVFGKELKVGSREAAFTYAIIAAGVAHAITAACTQGNLSDCGCDKEKQGQYHRDEGWKWGGCSADIRYGIGFAKVFVDAREIKQNARTLMNLHNNEAGRKILEENMKLECKCHGVSGSCTTKTCWTTLPQFRELGYVLADKYNEAVHVEPVRASRNKRPTFLKIKKPLSYRKPMDTDLVYIEKSPNYC

SEQ ID NO: 42 - protein, 247 aa, synthetic construct
  SOURCE 1..247
  REGION 1..247: NOTE = human N-terminal domain (NTD) Wnt7a variant V205A
LGASIICNKIPGLAPRQRAICQSRPDAIIVIGEGSQMGLDECQFQFRNGRWNCSALGERTVFGKELKVGSREAAFTYAIIAAGVAHAITAACTQGNLSDCGCDKEKQGQYHRDEGWKWGGCSADIRYGIGFAKVFVDAREIKQNARTLMNLHNNEAGRKILEENMKLECKCHGVSGSCTTKTCWTTLPQFRELGYVLKDKYNEAAHVEPVRASRNKRPTFLKIKKPLSYRKPMDTDLVYIEKSPNYC

SEQ ID NO: 43 - protein, 247 aa, synthetic construct
  SOURCE 1..247
  REGION 1..247: NOTE = human N-terminal domain (NTD) Wnt7a variant E208A
LGASIICNKIPGLAPRQRAICQSRPDAIIVIGEGSQMGLDECQFQFRNGRWNCSALGERTVFGKELKVGSREAAFTYAIIAAGVAHAITAACTQGNLSDCGCDKEKQGQYHRDEGWKWGGCSADIRYGIGFAKVFVDAREIKQNARTLMNLHNNEAGRKILEENMKLECKCHGVSGSCTTKTCWTTLPQFRELGYVLKDKYNEAVHVAPVRASRNKRPTFLKIKKPLSYRKPMDTDLVYIEKSPNYC

SEQ ID NO: 44 - protein, 247 aa, synthetic construct
  SOURCE 1..247
  REGION 1..247: NOTE = human N-terminal domain (NTD) Wnt7a variant K216A
LGASIICNKIPGLAPRQRAICQSRPDAIIVIGEGSQMGLDECQFQFRNGRWNCSALGERTVFGKELKVGSREAAFTYAIIAAGVAHAITAACTQGNLSDCGCDKEKQGQYHRDEGWKWGGCSADIRYGIGFAKVFVDAREIKQNARTLMNLHNNEAGRKILEENMKLECKCHGVSGSCTTKTCWTTLPQFRELGYVLKDKYNEAVHVEPVRASRNARPTFLKIKKPLSYRKPMDTDLVYIEKSPNYC

SEQ ID NO: 45 - protein, 247 aa, synthetic construct
  SOURCE 1..247
  REGION 1..247: NOTE = human N-terminal domain (NTD) Wnt7a variant K222A
LGASIICNKIPGLAPRQRAICQSRPDAIIVIGEGSQMGLDECQFQFRNGRWNCSALGERTVFGKELKVGSREAAFTYAIIAAGVAHAITAACTQGNLSDCGCDKEKQGQYHRDEGWKWGGCSADIRYGIGFAKVFVDAREIKQNARTLMNLHNNEAGRKILEENMKLECKCHGVSGSCTTKTCWTTLPQFRELGYVLKDKYNEAVHVEPVRASRNKRPTFLAIKKPLSYRKPMDTDLVYIEKSPNYC

SEQ ID NO: 46 - protein, 247 aa, synthetic construct
  SOURCE 1..247
  REGION 1..247: NOTE = human N-terminal domain (NTD) Wnt7a variant I223A
LGASIICNKIPGLAPRQRAICQSRPDAIIVIGEGSQMGLDECQFQFRNGRWNCSALGERTVFGKELKVGSREAAFTYAIIAAGVAHAITAACTQGNLSDCGCDKEKQGQYHRDEGWKWGGCSADIRYGIGFAKVFVDAREIKQNARTLMNLHNNEAGRKILEENMKLECKCHGVSGSCTTKTCWTTLPQFRELGYVLKDKYNEAVHVEPVRASRNKRPTFLKAKKPLSYRKPMDTDLVYIEKSPNYC

SEQ ID NO: 47 - protein, 247 aa, synthetic construct
  SOURCE 1..247
  REGION 1..247: NOTE = human N-terminal domain (NTD) Wnt7a variant Y229A
LGASIICNKIPGLAPRQRAICQSRPDAIIVIGEGSQMGLDECQFQFRNGRWNCSALGERTVFGKELKVGSREAAFTYAIIAAGVAHAITAACTQGNLSDCGCDKEKQGQYHRDEGWKWGGCSADIRYGIGFAKVFVDAREIKQNARTLMNLHNNEAGRKILEENMKLECKCHGVSGSCTTKTCWTTLPQFRELGYVLKDKYNEAVHVEPVRASRNKRPTFLKIKKPLSARKPMDTDLVYIEKSPNYC

SEQ ID NO: 48 - protein, 247 aa, synthetic construct
  SOURCE 1..247
  REGION 1..247: NOTE = human N-terminal domain (NTD) Wnt7a variant P232A
LGASIICNKIPGLAPRQRAICQSRPDAIIVIGEGSQMGLDECQFQFRNGRWNCSALGERTVFGKELKVGSREAAFTYAIIAAGVAHAITAACTQGNLSDCGCDKEKQGQYHRDEGWKWGGCSADIRYGIGFAKVFVDAREIKQNARTLMNLHNNEAGRKILEENMKLECKCHGVSGSCTTKTCWTTLPQFRELGYVLKDKYNEAVHVEPVRASRNKRPTFLKIKKPLSYRKAMDTDLVYIEKSPNYC

SEQ ID NO: 49 - protein, 247 aa, synthetic construct
  SOURCE 1..247
  REGION 1..247: NOTE = human N-terminal domain (NTD) Wnt7a variant T235A
LGASIICNKIPGLAPRQRAICQSRPDAIIVIGEGSQMGLDECQFQFRNGRWNCSALGERTVFGKELKVGSREAAFTYAIIAAGVAHAITAACTQGNLSDCGCDKEKQGQYHRDEGWKWGGCSADIRYGIGFAKVFVDAREIKQNARTLMNLHNNEAGRKILEENMKLECKCHGVSGSCTTKTCWTTLPQFRELGYVLKDKYNEAVHVEPVRASRNKRPTFLKIKKPLSYRKPMDADLVYIEKSPNYC

SEQ ID NO: 50 - protein, 318 aa, synthetic construct
  SOURCE 1..318
  REGION 1..318: NOTE = human full Wnt7a variant E248A
LGASIICNKIPGLAPRQRAICQSRPDAIIVIGEGSQMGLDECQFQFRNGRWNCSALGERTVFGKELKVGSREAAFTYAIIAAGVAHAITAACTQGNLSDCGCDKEKQGQYHRDEGWKWGGCSADIRYGIGFAKVFVDAREIKQNARTLMNLHNNEAGRKILEENMKLECKCHGVSGSCTTKTCWTTLPQFRELGYVLKDKYNEAVHVEPVRASRNKRPTFLKIKKPLSYRKPMDTDLVYIEKSPNYCAEDPVTGSVGTQGRACNKTAPQASGCDLMCCGRGYNTHQYARVWQCNCKFHWCCYVKCNTCSERTEMYTCK

SEQ ID NO: 51 - protein, 318 aa, Homo sapiens
  SOURCE 1..318
LGASIICNKIPGLAPRQRAICQSRPDAIIVIGEGSQMGLDECQFQFRNGRWNCSALGERTVFGKELKVGSREAAFTYAIIAAGVAHAITAACTQGNLSDCGCDKEKQGQYHRDEGWKWGGCSADIRYGIGFAKVFVDAREIKQNARTLMNLHNNEAGRKILEENMKLECKCHGVSGSCTTKTCWTTLPQFRELGYVLKDKYNEAVHVEPVRASRNKRPTFLKIKKPLSYRKPMDTDLVYIEKSPNYCEEDPVTGSVGTQGRACNKTAPQASGCDLMCCGRGYNTHQYARVWQCNCKFHWCCYVKCNTCSERTEMYTCK

SEQ ID NO: 52 - protein, 318 aa, synthetic construct
  SOURCE 1..318
  REGION 1..318: NOTE = human full Wnt7a variant R289A
LGASIICNKIPGLAPRQRAICQSRPDAIIVIGEGSQMGLDECQFQFRNGRWNCSALGERTVFGKELKVGSREAAFTYAIIAAGVAHAITAACTQGNLSDCGCDKEKQGQYHRDEGWKWGGCSADIRYGIGFAKVFVDAREIKQNARTLMNLHNNEAGRKILEENMKLECKCHGVSGSCTTKTCWTTLPQFRELGYVLKDKYNEAVHVEPVRASRNKRPTFLKIKKPLSYRKPMDTDLVYIEKSPNYCEEDPVTGSVGTQGRACNKTAPQASGCDLMCCGRGYNTHQYAAVWQCNCKFHWCCYVKCNTCSERTEMYTCK

SEQ ID NO: 53 - protein, 318 aa, synthetic construct
  SOURCE 1..318
  REGION 1..318: NOTE = human full Wnt7a variant W291A
LGASIICNKIPGLAPRQRAICQSRPDAIIVIGEGSQMGLDECQFQFRNGRWNCSALGERTVFGKELKVGSREAAFTYAIIAAGVAHAITAACTQGNLSDCGCDKEKQGQYHRDEGWKWGGCSADIRYGIGFAKVFVDAREIKQNARTLMNLHNNEAGRKILEENMKLECKCHGVSGSCTTKTCWTTLPQFRELGYVLKDKYNEAVHVEPVRASRNKRPTFLKIKKPLSYRKPMDTDLVYIEKSPNYCEEDPVTGSVGTQGRACNKTAPQASGCDLMCCGRGYNTHQYARVAQCNCKFHWCCYVKCNTCSERTEMYTCK

SEQ ID NO: 54 - protein, 318 aa, synthetic construct
  SOURCE 1..318
  REGION 1..318: NOTE = human full Wnt7a variant T307A
LGASIICNKIPGLAPRQRAICQSRPDAIIVIGEGSQMGLDECQFQFRNGRWNCSALGERTVFGKELKVGSREAAFTYAIIAAGVAHAITAACTQGNLSDCGCDKEKQGQYHRDEGWKWGGCSADIRYGIGFAKVFVDAREIKQNARTLMNLHNNEAGRKILEENMKLECKCHGVSGSCTTKTCWTTLPQFRELGYVLKDKYNEAVHVEPVRASRNKRPTFLKIKKPLSYRKPMDTDLVYIEKSPNYCEEDPVTGSVGTQGRACNKTAPQASGCDLMCCGRGYNTHQYARVWQCNCKFHWCCYVKCNACSERTEMYTCK

SEQ ID NO: 55 - protein, 11 aa, synthetic construct
  SOURCE 1..11
  REGION 1..11: NOTE = peptide displayed on AAV-PHP.B
SAQTLAVPFKA

SEQ ID NO: 56 - protein, 11 aa, synthetic construct
  SOURCE 1..11
  REGION 1..11: NOTE = peptide displayed on AAV-PHP.eB
SDGTLAVPFKA

SEQ ID NO: 57 - protein, 7 aa, synthetic construct
  SOURCE 1..7
  REGION 1..7: NOTE = peptide displayed on AAV-BR1
NRGTEWD

SEQ ID NO: 58 - protein, 27 aa, synthetic construct
  SOURCE 1..27
  REGION 1..27: NOTE = xenopus Levis
VEPVRASRNKRPTFLKIKNSYRKPMDT

SEQ ID NO: 59 - protein, 29 aa, synthetic construct
  SOURCE 1..29
  REGION 1..29: NOTE = danio rerio
VEPVRASRNKRPAFLKVKKPYSYRKPMDT

SEQ ID NO: 60 - protein, 29 aa, synthetic construct
  SOURCE 1..29
  REGION 1..29: NOTE = danio rerio
VEPVKATRHKRPTFLKIKKPYSYRKPMDT

SEQ ID NO: 61 - protein, 29 aa, synthetic construct
  SOURCE 1..29
  REGION 1..29: NOTE = mus musculus
VEVVRASRLRQPTFLRIKQLRSYQKPMET

SEQ ID NO: 62 - protein, 29 aa, synthetic construct
  SOURCE 1..29
  REGION 1..29: NOTE = gallus gallus
VEVVRASRLRQPTFLKIKQIKSYQKPMET

SEQ ID NO: 63 - protein, 29 aa, synthetic construct
  SOURCE 1..29
  REGION 1..29: NOTE = xenopus Levis
VEVVRANRLRQPTFLKIKKVRSYQKPMET

SEQ ID NO: 64 - protein, 28 aa, synthetic construct
  SOURCE 1..28
  REGION 1..28: NOTE = Danio rerio
VEVVRASRLRQPTFLKVKRTRHQKPLET

SEQ ID NO: 65 - protein, 29 aa, synthetic construct
  SOURCE 1..29
  REGION 1..29: NOTE = Danio rerio
VEAVRATRFRQPSFLRLKQSRGYIKPTDT

SEQ ID NO: 66 - protein, 29 aa, synthetic construct
  SOURCE 1..29
  REGION 1..29: NOTE = mus musculus
MVVEKHRESRGWVETLRPRYTYFKVPTER

SEQ ID NO: 67 - protein, 29 aa, synthetic construct
  SOURCE 1..29
  REGION 1..29: NOTE = quadruple pWnt7a4A variant
VEPARASRNKRPTAAKIKKPLSYRAPMDT

SEQ ID NO: 68 - protein, 247 aa, synthetic construct
  SOURCE 1..247
  REGION 1..247: NOTE = human N-terminal domain (NTD) Wnt7a variant Q17A
LGASIICNKIPGLAPRARAICQSRPDAIIVIGEGSQMGLDECQFQFRNGRWNCSALGERTVFGKELKVGSREAAFTYAIIAAGVAHAITAACTQGNLSDCGCDKEKQGQYHRDEGWKWGGCSADIRYGIGFAKVFVDAREIKQNARTLMNLHNNEAGRKILEENMKLECKCHGVSGSCTTKTCWTTLPQFRELGYVLKDKYNEAVHVEPVRASRNKRPTFLKIKKPLSYRKPMDTDLVYIEKSPNYC

SEQ ID NO: 69 - protein, 247 aa, synthetic construct
  SOURCE 1..247
  REGION 1..247: NOTE = human N-terminal domain (NTD) Wnt7a variant I20A
LGASIICNKIPGLAPRQRAACQSRPDAIIVIGEGSQMGLDECQFQFRNGRWNCSALGERTVFGKELKVGSREAAFTYAIIAAGVAHAITAACTQGNLSDCGCDKEKQGQYHRDEGWKWGGCSADIRYGIGFAKVFVDAREIKQNARTLMNLHNNEAGRKILEENMKLECKCHGVSGSCTTKTCWTTLPQFRELGYVLKDKYNEAVHVEPVRASRNKRPTFLKIKKPLSYRKPMDTDLVYIEKSPNYC

SEQ ID NO: 70 - protein, 247 aa, synthetic construct
  SOURCE 1..247
  REGION 1..247: NOTE = human N-terminal domain (NTD) Wnt7a variant P25A
LGASIICNKIPGLAPRQRAICQSRADAIIVIGEGSQMGLDECQFQFRNGRWNCSALGERTVFGKELKVGSREAAFTYAIIAAGVAHAITAACTQGNLSDCGCDKEKQGQYHRDEGWKWGGCSADIRYGIGFAKVFVDAREIKQNARTLMNLHNNEAGRKILEENMKLECKCHGVSGSCTTKTCWTTLPQFRELGYVLKDKYNEAVHVEPVRASRNKRPTFLKIKKPLSYRKPMDTDLVYIEKSPNYC

SEQ ID NO: 71 - protein, 247 aa, synthetic construct
  SOURCE 1..247
  REGION 1..247: NOTE = human N-terminal domain (NTD) Wnt7a variant M37A
LGASIICNKIPGLAPRQRAICQSRPDAIIVIGEGSQAGLDECQFQFRNGRWNCSALGERTVFGKELKVGSREAAFTYAIIAAGVAHAITAACTQGNLSDCGCDKEKQGQYHRDEGWKWGGCSADIRYGIGFAKVFVDAREIKQNARTLMNLHNNEAGRKILEENMKLECKCHGVSGSCTTKTCWTTLPQFRELGYVLKDKYNEAVHVEPVRASRNKRPTFLKIKKPLSYRKPMDTDLVYIEKSPNYC

SEQ ID NO: 72 - protein, 247 aa, synthetic construct
  SOURCE 1..247
  REGION 1..247: NOTE = human N-terminal domain (NTD) Wnt7a variant L39A
LGASIICNKIPGLAPRQRAICQSRPDAIIVIGEGSQMGADECQFQFRNGRWNCSALGERTVFGKELKVGSREAAFTYAIIAAGVAHAITAACTQGNLSDCGCDKEKQGQYHRDEGWKWGGCSADIRYGIGFAKVFVDAREIKQNARTLMNLHNNEAGRKILEENMKLECKCHGVSGSCTTKTCWTTLPQFRELGYVLKDKYNEAVHVEPVRASRNKRPTFLKIKKPLSYRKPMDTDLVYIEKSPNYC

SEQ ID NO: 73 - DNA, 25 bp, synthetic construct
  source 1..25: mol_type = other DNA
  misc_feature 1..25: note = wnt7aa Morpholino
ttccatttgaccctacttacccaat

SEQ ID NO: 74 - protein, 247 aa, synthetic construct
  SOURCE 1..247
  REGION 1..247: NOTE = human N-terminal domain (NTD) Wnt7a variant I28A
LGASIICNKIPGLAPRQRAICQSRPDAAIVIGEGSQMGLDECQFQFRNGRWNCSALGERTVFGKELKVGSREAAFTYAIIAAGVAHAITAACTQGNLSDCGCDKEKQGQYHRDEGWKWGGCSADIRYGIGFAKVFVDAREIKQNARTLMNLHNNEAGRKILEENMKLECKCHGVSGSCTTKTCWTTLPQFRELGYVLKDKYNEAVHVEPVRASRNKRPTFLKIKKPLSYRKPMDTDLVYIEKSPNYC

SEQ ID NO: 75 - protein, 247 aa, synthetic construct
  SOURCE 1..247
  REGION 1..247: NOTE = human N-terminal domain (NTD) Wnt7a variant R50A
LGASIICNKIPGLAPRQRAICQSRPDAIIVIGEGSQMGLDECQFQFRNGAWNCSALGERTVFGKELKVGSREAAFTYAIIAAGVAHAITAACTQGNLSDCGCDKEKQGQYHRDEGWKWGGCSADIRYGIGFAKVFVDAREIKQNARTLMNLHNNEAGRKILEENMKLECKCHGVSGSCTTKTCWTTLPQFRELGYVLKDKYNEAVHVEPVRASRNKRPTFLKIKKPLSYRKPMDTDLVYIEKSPNYC

SEQ ID NO: 76 - protein, 247 aa, synthetic construct
  SOURCE 1..247
  REGION 1..247: NOTE = human N-terminal domain (NTD) Wnt7a variant V68A
LGASIICNKIPGLAPRQRAICQSRPDAIIVIGEGSQMGLDECQFQFRNGRWNCSALGERTVFGKELKAGSREAAFTYAIIAAGVAHAITAACTQGNLSDCGCDKEKQGQYHRDEGWKWGGCSADIRYGIGFAKVFVDAREIKQNARTLMNLHNNEAGRKILEENMKLECKCHGVSGSCTTKTCWTTLPQFRELGYVLKDKYNEAVHVEPVRASRNKRPTFLKIKKPLSYRKPMDTDLVYIEKSPNYC

SEQ ID NO: 77 - protein, 247 aa, synthetic construct
  SOURCE 1..247
  REGION 1..247: NOTE = human N-terminal domain (NTD) Wnt7a variant F135A
LGASIICNKIPGLAPRQRAICQSRPDAIIVIGEGSQMGLDECQFQFRNGRWNCSALGERTVFGKELKVGSREAAFTYAIIAAGVAHAITAACTQGNLSDCGCDKEKQGQYHRDEGWKWGGCSADIRYGIGFAKVAVDAREIKQNARTLMNLHNNEAGRKILEENMKLECKCHGVSGSCTTKTCWTTLPQFRELGYVLKDKYNEAVHVEPVRASRNKRPTFLKIKKPLSYRKPMDTDLVYIEKSPNYC

SEQ ID NO: 78 - protein, 247 aa, synthetic construct
  SOURCE 1..247
  REGION 1..247: NOTE = human N-terminal domain (NTD) Wnt7a variant R146A
LGASIICNKIPGLAPRQRAICQSRPDAIIVIGEGSQMGLDECQFQFRNGRWNCSALGERTVFGKELKVGSREAAFTYAIIAAGVAHAITAACTQGNLSDCGCDKEKQGQYHRDEGWKWGGCSADIRYGIGFAKVFVDAREIKQNAATLMNLHNNEAGRKILEENMKLECKCHGVSGSCTTKTCWTTLPQFRELGYVLKDKYNEAVHVEPVRASRNKRPTFLKIKKPLSYRKPMDTDLVYIEKSPNYC

SEQ ID NO: 79 - protein, 247 aa, synthetic construct
  SOURCE 1..247
  REGION 1..247: NOTE = human N-terminal domain (NTD) Wnt7a variant K159S
LGASIICNKIPGLAPRQRAICQSRPDAIIVIGEGSQMGLDECQFQFRNGRWNCSALGERTVFGKELKVGSREAAFTYAIIAAGVAHAITAACTQGNLSDCGCDKEKQGQYHRDEGWKWGGCSADIRYGIGFAKVFVDAREIKQNARTLMNLHNNEAGRSILEENMKLECKCHGVSGSCTTKTCWTTLPQFRELGYVLKDKYNEAVHVEPVRASRNKRPTFLKIKKPLSYRKPMDTDLVYIEKSPNYC

SEQ ID NO: 80 - protein, 247 aa, synthetic construct
  SOURCE 1..247
  REGION 1..247: NOTE = human N-terminal domain (NTD) Wnt7a variant K159L
LGASIICNKIPGLAPRQRAICQSRPDAIIVIGEGSQMGLDECQFQFRNGRWNCSALGERTVFGKELKVGSREAAFTYAIIAAGVAHAITAACTQGNLSDCGCDKEKQGQYHRDEGWKWGGCSADIRYGIGFAKVFVDAREIKQNARTLMNLHNNEAGRLILEENMKLECKCHGVSGSCTTKTCWTTLPQFRELGYVLKDKYNEAVHVEPVRASRNKRPTFLKIKKPLSYRKPMDTDLVYIEKSPNYC

SEQ ID NO: 81 - protein, 247 aa, synthetic construct
  SOURCE 1..247
  REGION 1..247: NOTE = human N-terminal domain (NTD) Wnt7a variant K200A
LGASIICNKIPGLAPRQRAICQSRPDAIIVIGEGSQMGLDECQFQFRNGRWNCSALGERTVFGKELKVGSREAAFTYAIIAAGVAHAITAACTQGNLSDCGCDKEKQGQYHRDEGWKWGGCSADIRYGIGFAKVFVDAREIKQNARTLMNLHNNEAGRKILEENMKLECKCHGVSGSCTTKTCWTTLPQFRELGYVLKDAYNEAVHVEPVRASRNKRPTFLKIKKPLSYRKPMDTDLVYIEKSPNYC

SEQ ID NO: 82 - protein, 247 aa, synthetic construct
  SOURCE 1..247
  REGION 1..247: NOTE = human N-terminal domain (NTD) Wnt7a variant R214A
LGASIICNKIPGLAPRQRAICQSRPDAIIVIGEGSQMGLDECQFQFRNGRWNCSALGERTVFGKELKVGSREAAFTYAIIAAGVAHAITAACTQGNLSDCGCDKEKQGQYHRDEGWKWGGCSADIRYGIGFAKVFVDAREIKQNARTLMNLHNNEAGRKILEENMKLECKCHGVSGSCTTKTCWTTLPQFRELGYVLKDKYNEAVHVEPVRASANKRPTFLKIKKPLSYRKPMDTDLVYIEKSPNYC

SEQ ID NO: 83 - protein, 247 aa, synthetic construct; identical to SEQ ID NO: 24
  SOURCE 1..247
  REGION 1..247: NOTE = human N-terminal domain (NTD) Wnt7a variant P218A

SEQ ID NO: 84 - protein, 318 aa, synthetic construct
  SOURCE 1..318
  REGION 1..318: NOTE = human Wnt7a variant K318A
LGASIICNKIPGLAPRQRAICQSRPDAIIVIGEGSQMGLDECQFQFRNGRWNCSALGERTVFGKELKVGSREAAFTYAIIAAGVAHAITAACTQGNLSDCGCDKEKQGQYHRDEGWKWGGCSADIRYGIGFAKVFVDAREIKQNARTLMNLHNNEAGRKILEENMKLECKCHGVSGSCTTKTCWTTLPQFRELGYVLKDKYNEAVHVEPVRASRNKRPTFLKIKKPLSYRKPMDTDLVYIEKSPNYCEEDPVTGSVGTQGRACNKTAPQASGCDLMCCGRGYNTHQYARVWQCNCKFHWCCYVKCNTCSERTEMYTCA

SEQ ID NO: 85 - protein, 318 aa, synthetic construct
  SOURCE 1..318
  REGION 1..318: NOTE = human Wnt7a variant K159A
LGASIICNKIPGLAPRQRAICQSRPDAIIVIGEGSQMGLDECQFQFRNGRWNCSALGERTVFGKELKVGSREAAFTYAIIAAGVAHAITAACTQGNLSDCGCDKEKQGQYHRDEGWKWGGCSADIRYGIGFAKVFVDAREIKQNARTLMNLHNNEAGRAILEENMKLECKCHGVSGSCTTKTCWTTLPQFRELGYVLKDKYNEAVHVEPVRASRNKRPTFLKIKKPLSYRKPMDTDLVYIEKSPNYCEEDPVTGSVGTQGRACNKTAPQASGCDLMCCGRGYNTHQYARVWQCNCKFHWCCYVKCNTCSERTEMYTCK

SEQ ID NO: 86 - protein, 318 aa, synthetic construct
  SOURCE 1..318
  REGION 1..318: NOTE = human Wnt7a variant A27R
LGASIICNKIPGLAPRQRAICQSRPDRIIVIGEGSQMGLDECQFQFRNGRWNCSALGERTVFGKELKVGSREAAFTYAIIAAGVAHAITAACTQGNLSDCGCDKEKQGQYHRDEGWKWGGCSADIRYGIGFAKVFVDAREIKQNARTLMNLHNNEAGRKILEENMKLECKCHGVSGSCTTKTCWTTLPQFRELGYVLKDKYNEAVHVEPVRASRNKRPTFLKIKKPLSYRKPMDTDLVYIEKSPNYCEEDPVTGSVGTQGRACNKTAPQASGCDLMCCGRGYNTHQYARVWQCNCKFHWCCYVKCNTCSERTEMYTCK

SEQ ID NO: 87 - protein, 318 aa, synthetic construct
  SOURCE 1..318
  REGION 1..318: NOTE = human Wnt7a variant E33A
LGASIICNKIPGLAPRQRAICQSRPDAIIVIGAGSQMGLDECQFQFRNGRWNCSALGERTVFGKELKVGSREAAFTYAIIAAGVAHAITAACTQGNLSDCGCDKEKQGQYHRDEGWKWGGCSADIRYGIGFAKVFVDAREIKQNARTLMNLHNNEAGRKILEENMKLECKCHGVSGSCTTKTCWTTLPQFRELGYVLKDKYNEAVHVEPVRASRNKRPTFLKIKKPLSYRKPMDTDLVYIEKSPNYCEEDPVTGSVGTQGRACNKTAPQASGCDLMCCGRGYNTHQYARVWQCNCKFHWCCYVKCNTCSERTEMYTCK

SEQ ID NO: 88 - protein, 318 aa, synthetic construct
  SOURCE 1..318
  REGION 1..318: NOTE = human Wnt7a variant E41A
LGASIICNKIPGLAPRQRAICQSRPDAIIVIGEGSQMGLDACQFQFRNGRWNCSALGERTVFGKELKVGSREAAFTYAIIAAGVAHAITAACTQGNLSDCGCDKEKQGQYHRDEGWKWGGCSADIRYGIGFAKVFVDAREIKQNARTLMNLHNNEAGRKILEENMKLECKCHGVSGSCTTKTCWTTLPQFRELGYVLKDKYNEAVHVEPVRASRNKRPTFLKIKKPLSYRKPMDTDLVYIEKSPNYCEEDPVTGSVGTQGRACNKTAPQASGCDLMCCGRGYNTHQYARVWQCNCKFHWCCYVKCNTCSERTEMYTCK

SEQ ID NO: 89 - protein, 318 aa, synthetic construct
  SOURCE 1..318
  REGION 1..318: NOTE = human Wnt7a variant F44A
LGASIICNKIPGLAPRQRAICQSRPDAIIVIGEGSQMGLDECQAQFRNGRWNCSALGERTVFGKELKVGSREAAFTYAIIAAGVAHAITAACTQGNLSDCGCDKEKQGQYHRDEGWKWGGCSADIRYGIGFAKVFVDAREIKQNARTLMNLHNNEAGRKILEENMKLECKCHGVSGSCTTKTCWTTLPQFRELGYVLKDKYNEAVHVEPVRASRNKRPTFLKIKKPLSYRKPMDTDLVYIEKSPNYCEEDPVTGSVGTQGRACNKTAPQASGCDLMCCGRGYNTHQYARVWQCNCKFHWCCYVKCNTCSERTEMYTCK

SEQ ID NO: 90 - protein, 318 aa, synthetic construct
  SOURCE 1..318
  REGION 1..318: NOTE = human Wnt7a variant N52Q
LGASIICNKIPGLAPRQRAICQSRPDAIIVIGEGSQMGLDECQFQFRNGRWQCSALGERTVFGKELKVGSREAAFTYAIIAAGVAHAITAACTQGNLSDCGCDKEKQGQYHRDEGWKWGGCSADIRYGIGFAKVFVDAREIKQNARTLMNLHNNEAGRKILEENMKLECKCHGVSGSCTTKTCWTTLPQFRELGYVLKDKYNEAVHVEPVRASRNKRPTFLKIKKPLSYRKPMDTDLVYIEKSPNYCEEDPVTGSVGTQGRACNKTAPQASGCDLMCCGRGYNTHQYARVWQCNCKFHWCCYVKCNTCSERTEMYTCK

SEQ ID NO: 91 - protein, 318 aa, synthetic construct
  SOURCE 1..318
  REGION 1..318: NOTE = human Wnt7a variant I129A
LGASIICNKIPGLAPRQRAICQSRPDAIIVIGEGSQMGLDECQFQFRNGRWNCSALGERTVFGKELKVGSREAAFTYAIIAAGVAHAITAACTQGNLSDCGCDKEKQGQYHRDEGWKWGGCSADIRYGAGFAKVFVDAREIKQNARTLMNLHNNEAGRKILEENMKLECKCHGVSGSCTTKTCWTTLPQFRELGYVLKDKYNEAVHVEPVRASRNKRPTFLKIKKPLSYRKPMDTDLVYIEKSPNYCEEDPVTGSVGTQGRACNKTAPQASGCDLMCCGRGYNTHQYARVWQCNCKFHWCCYVKCNTCSERTEMYTCK

SEQ ID NO: 92 - protein, 318 aa, synthetic construct
  SOURCE 1..318
  REGION 1..318: NOTE = human Wnt7a variant F131A
LGASIICNKIPGLAPRQRAICQSRPDAIIVIGEGSQMGLDECQFQFRNGRWNCSALGERTVFGKELKVGSREAAFTYAIIAAGVAHAITAACTQGNLSDCGCDKEKQGQYHRDEGWKWGGCSADIRYGIGAAKVFVDAREIKQNARTLMNLHNNEAGRKILEENMKLECKCHGVSGSCTTKTCWTTLPQFRELGYVLKDKYNEAVHVEPVRASRNKRPTFLKIKKPLSYRKPMDTDLVYIEKSPNYCEEDPVTGSVGTQGRACNKTAPQASGCDLMCCGRGYNTHQYARVWQCNCKFHWCCYVKCNTCSERTEMYTCK

SEQ ID NO: 93 - protein, 318 aa, synthetic construct
  SOURCE 1..318
  REGION 1..318: NOTE = human Wnt7a variant K133A
LGASIICNKIPGLAPRQRAICQSRPDAIIVIGEGSQMGLDECQFQFRNGRWNCSALGERTVFGKELKVGSREAAFTYAIIAAGVAHAITAACTQGNLSDCGCDKEKQGQYHRDEGWKWGGCSADIRYGIGFAAVFVDAREIKQNARTLMNLHNNEAGRKILEENMKLECKCHGVSGSCTTKTCWTTLPQFRELGYVLKDKYNEAVHVEPVRASRNKRPTFLKIKKPLSYRKPMDTDLVYIEKSPNYCEEDPVTGSVGTQGRACNKTAPQASGCDLMCCGRGYNTHQYARVWQCNCKFHWCCYVKCNTCSERTEMYTCK

SEQ ID NO: 94 - protein, 318 aa, synthetic construct
  SOURCE 1..318
  REGION 1..318: NOTE = human Wnt7a variant I141A
LGASIICNKIPGLAPRQRAICQSRPDAIIVIGEGSQMGLDECQFQFRNGRWNCSALGERTVFGKELKVGSREAAFTYAIIAAGVAHAITAACTQGNLSDCGCDKEKQGQYHRDEGWKWGGCSADIRYGIGFAKVFVDAREAKQNARTLMNLHNNEAGRKILEENMKLECKCHGVSGSCTTKTCWTTLPQFRELGYVLKDKYNEAVHVEPVRASRNKRPTFLKIKKPLSYRKPMDTDLVYIEKSPNYCEEDPVTGSVGTQGRACNKTAPQASGCDLMCCGRGYNTHQYARVWQCNCKFHWCCYVKCNTCSERTEMYTCK

SEQ ID NO: 95 - protein, 318 aa, synthetic construct
  SOURCE 1..318
  REGION 1..318: NOTE = human Wnt7a variant R158A
LGASIICNKIPGLAPRQRAICQSRPDAIIVIGEGSQMGLDECQFQFRNGRWNCSALGERTVFGKELKVGSREAAFTYAIIAAGVAHAITAACTQGNLSDCGCDKEKQGQYHRDEGWKWGGCSADIRYGIGFAKVFVDAREIKQNARTLMNLHNNEAGAKILEENMKLECKCHGVSGSCTTKTCWTTLPQFRELGYVLKDKYNEAVHVEPVRASRNKRPTFLKIKKPLSYRKPMDTDLVYIEKSPNYCEEDPVTGSVGTQGRACNKTAPQASGCDLMCCGRGYNTHQYARVWQCNCKFHWCCYVKCNTCSERTEMYTCK

SEQ ID NO: 96 - protein, 318 aa, synthetic construct
  SOURCE 1..318
  REGION 1..318: NOTE = human Wnt7a variant K181A
LGASIICNKIPGLAPRQRAICQSRPDAIIVIGEGSQMGLDECQFQFRNGRWNCSALGERTVFGKELKVGSREAAFTYAIIAAGVAHAITAACTQGNLSDCGCDKEKQGQYHRDEGWKWGGCSADIRYGIGFAKVFVDAREIKQNARTLMNLHNNEAGRKILEENMKLECKCHGVSGSCTTATCWTTLPQFRELGYVLKDKYNEAVHVEPVRASRNKRPTFLKIKKPLSYRKPMDTDLVYIEKSPNYCEEDPVTGSVGTQGRACNKTAPQASGCDLMCCGRGYNTHQYARVWQCNCKFHWCCYVKCNTCSERTEMYTCK

SEQ ID NO: 97 - protein, 318 aa, synthetic construct
  SOURCE 1..318
  REGION 1..318: NOTE = human Wnt7a variant R191A
LGASIICNKIPGLAPRQRAICQSRPDAIIVIGEGSQMGLDECQFQFRNGRWNCSALGERTVFGKELKVGSREAAFTYAIIAAGVAHAITAACTQGNLSDCGCDKEKQGQYHRDEGWKWGGCSADIRYGIGFAKVFVDAREIKQNARTLMNLHNNEAGRKILEENMKLECKCHGVSGSCTTKTCWTTLPQFAELGYVLKDKYNEAVHVEPVRASRNKRPTFLKIKKPLSYRKPMDTDLVYIEKSPNYCEEDPVTGSVGTQGRACNKTAPQASGCDLMCCGRGYNTHQYARVWQCNCKFHWCCYVKCNTCSERTEMYTCK

SEQ ID NO: 98 - protein, 318 aa, synthetic construct
  SOURCE 1..318
  REGION 1..318: NOTE = human Wnt7a variant K198A
LGASIICNKIPGLAPRQRAICQSRPDAIIVIGEGSQMGLDECQFQFRNGRWNCSALGERTVFGKELKVGSREAAFTYAIIAAGVAHAITAACTQGNLSDCGCDKEKQGQYHRDEGWKWGGCSADIRYGIGFAKVFVDAREIKQNARTLMNLHNNEAGRKILEENMKLECKCHGVSGSCTTKTCWTTLPQFRELGYVLADKYNEAVHVEPVRASRNKRPTFLKIKKPLSYRKPMDTDLVYIEKSPNYCEEDPVTGSVGTQGRACNKTAPQASGCDLMCCGRGYNTHQYARVWQCNCKFHWCCYVKCNTCSERTEMYTCK

SEQ ID NO: 99 - protein, 317 aa, synthetic construct
  SOURCE 1..317
  REGION 1..317: NOTE = human Wnt7a variant V205A
LGASIICNKIPGLAPRQRAICQSRPDAIIVIGEGSQMGLDECQFQFRNGRWNCSALGERTVFGKELKVGSREAAFTYAIIAAGVAHAITAACTQGNLSDCGCDKEKQGQYHRDEGWKWGGCSADIRYGIGFAKVFVDAREIKQNARTLMNLHNNEAGRKILEENMKLECKCHGVSGSCTTKTCWTTLPQFRELGYVLKDKYNEAAHVEPVRASRNKRPTFLKIKKPLSYRKPMDTDLVYIEKSPNYEEDPVTGSVGTQGRACNKTAPQASGCDLMCCGRGYNTHQYARVWQCNCKFHWCCYVKCNTCSERTEMYTCK

SEQ ID NO: 100 - protein, 318 aa, synthetic construct
  SOURCE 1..318
  REGION 1..318: NOTE = human Wnt7a variant E208A
LGASIICNKIPGLAPRQRAICQSRPDAIIVIGEGSQMGLDECQFQFRNGRWNCSALGERTVFGKELKVGSREAAFTYAIIAAGVAHAITAACTQGNLSDCGCDKEKQGQYHRDEGWKWGGCSADIRYGIGFAKVFVDAREIKQNARTLMNLHNNEAGRKILEENMKLECKCHGVSGSCTTKTCWTTLPQFRELGYVLKDKYNEAVHVAPVRASRNKRPTFLKIKKPLSYRKPMDTDLVYIEKSPNYCEEDPVTGSVGTQGRACNKTAPQASGCDLMCCGRGYNTHQYARVWQCNCKFHWCCYVKCNTCSERTEMYTCK

SEQ ID NO: 101 - protein, 318 aa, synthetic construct
  SOURCE 1..318
  REGION 1..318: NOTE = human Wnt7a variant K216A
LGASIICNKIPGLAPRQRAICQSRPDAIIVIGEGSQMGLDECQFQFRNGRWNCSALGERTVFGKELKVGSREAAFTYAIIAAGVAHAITAACTQGNLSDCGCDKEKQGQYHRDEGWKWGGCSADIRYGIGFAKVFVDAREIKQNARTLMNLHNNEAGRKILEENMKLECKCHGVSGSCTTKTCWTTLPQFRELGYVLKDKYNEAVHVEPVRASRNARPTFLKIKKPLSYRKPMDTDLVYIEKSPNYCEEDPVTGSVGTQGRACNKTAPQASGCDLMCCGRGYNTHQYARVWQCNCKFHWCCYVKCNTCSERTEMYTCK

SEQ ID NO: 102 - protein, 318 aa, synthetic construct
  SOURCE 1..318
  REGION 1..318: NOTE = human Wnt7a variant K222A
LGASIICNKIPGLAPRQRAICQSRPDAIIVIGEGSQMGLDECQFQFRNGRWNCSALGERTVFGKELKVGSREAAFTYAIIAAGVAHAITAACTQGNLSDCGCDKEKQGQYHRDEGWKWGGCSADIRYGIGFAKVFVDAREIKQNARTLMNLHNNEAGRKILEENMKLECKCHGVSGSCTTKTCWTTLPQFRELGYVLKDKYNEAVHVEPVRASRNKRPTFLAIKKPLSYRKPMDTDLVYIEKSPNYCEEDPVTGSVGTQGRACNKTAPQASGCDLMCCGRGYNTHQYARVWQCNCKFHWCCYVKCNTCSERTEMYTCK

SEQ ID NO: 103 - protein, 318 aa, synthetic construct
  SOURCE 1..318
  REGION 1..318: NOTE = human Wnt7a variant I223A
LGASIICNKIPGLAPRQRAICQSRPDAIIVIGEGSQMGLDECQFQFRNGRWNCSALGERTVFGKELKVGSREAAFTYAIIAAGVAHAITAACTQGNLSDCGCDKEKQGQYHRDEGWKWGGCSADIRYGIGFAKVFVDAREIKQNARTLMNLHNNEAGRKILEENMKLECKCHGVSGSCTTKTCWTTLPQFRELGYVLKDKYNEAVHVEPVRASRNKRPTFLKAKKPLSYRKPMDTDLVYIEKSPNYCEEDPVTGSVGTQGRACNKTAPQASGCDLMCCGRGYNTHQYARVWQCNCKFHWCCYVKCNTCSERTEMYTCK

SEQ ID NO: 104 - protein, 318 aa, synthetic construct
  SOURCE 1..318
  REGION 1..318: NOTE = human Wnt7a variant Y229A
LGASIICNKIPGLAPRQRAICQSRPDAIIVIGEGSQMGLDECQFQFRNGRWNCSALGERTVFGKELKVGSREAAFTYAIIAAGVAHAITAACTQGNLSDCGCDKEKQGQYHRDEGWKWGGCSADIRYGIGFAKVFVDAREIKQNARTLMNLHNNEAGRKILEENMKLECKCHGVSGSCTTKTCWTTLPQFRELGYVLKDKYNEAVHVEPVRASRNKRPTFLKIKKPLSARKPMDTDLVYIEKSPNYCEEDPVTGSVGTQGRACNKTAPQASGCDLMCCGRGYNTHQYARVWQCNCKFHWCCYVKCNTCSERTEMYTCK

SEQ ID NO: 105 - protein, 318 aa, synthetic construct
  SOURCE 1..318
  REGION 1..318: NOTE = human Wnt7a variant P232A
LGASIICNKIPGLAPRQRAICQSRPDAIIVIGEGSQMGLDECQFQFRNGRWNCSALGERTVFGKELKVGSREAAFTYAIIAAGVAHAITAACTQGNLSDCGCDKEKQGQYHRDEGWKWGGCSADIRYGIGFAKVFVDAREIKQNARTLMNLHNNEAGRKILEENMKLECKCHGVSGSCTTKTCWTTLPQFRELGYVLKDKYNEAVHVEPVRASRNKRPTFLKIKKPLSYRKAMDTDLVYIEKSPNYCEEDPVTGSVGTQGRACNKTAPQASGCDLMCCGRGYNTHQYARVWQCNCKFHWCCYVKCNTCSERTEMYTCK

SEQ ID NO: 106 - protein, 318 aa, synthetic construct
  SOURCE 1..318
  REGION 1..318: NOTE = human Wnt7a variant T235A
LGASIICNKIPGLAPRQRAICQSRPDAIIVIGEGSQMGLDECQFQFRNGRWNCSALGERTVFGKELKVGSREAAFTYAIIAAGVAHAITAACTQGNLSDCGCDKEKQGQYHRDEGWKWGGCSADIRYGIGFAKVFVDAREIKQNARTLMNLHNNEAGRKILEENMKLECKCHGVSGSCTTKTCWTTLPQFRELGYVLKDKYNEAVHVEPVRASRNKRPTFLKIKKPLSYRKPMDADLVYIEKSPNYCEEDPVTGSVGTQGRACNKTAPQASGCDLMCCGRGYNTHQYARVWQCNCKFHWCCYVKCNTCSERTEMYTCK

SEQ ID NO: 107 - protein, 318 aa, synthetic construct
  SOURCE 1..318
  REGION 1..318: NOTE = human Wnt7a variant Q17A
LGASIICNKIPGLAPRARAICQSRPDAIIVIGEGSQMGLDECQFQFRNGRWNCSALGERTVFGKELKVGSREAAFTYAIIAAGVAHAITAACTQGNLSDCGCDKEKQGQYHRDEGWKWGGCSADIRYGIGFAKVFVDAREIKQNARTLMNLHNNEAGRKILEENMKLECKCHGVSGSCTTKTCWTTLPQFRELGYVLKDKYNEAVHVEPVRASRNKRPTFLKIKKPLSYRKPMDTDLVYIEKSPNYCEEDPVTGSVGTQGRACNKTAPQASGCDLMCCGRGYNTHQYARVWQCNCKFHWCCYVKCNTCSERTEMYTCK

SEQ ID NO: 108 - protein, 318 aa, synthetic construct
  SOURCE 1..318
  REGION 1..318: NOTE = human Wnt7a variant I20A
LGASIICNKIPGLAPRQRAACQSRPDAIIVIGEGSQMGLDECQFQFRNGRWNCSALGERTVFGKELKVGSREAAFTYAIIAAGVAHAITAACTQGNLSDCGCDKEKQGQYHRDEGWKWGGCSADIRYGIGFAKVFVDAREIKQNARTLMNLHNNEAGRKILEENMKLECKCHGVSGSCTTKTCWTTLPQFRELGYVLKDKYNEAVHVEPVRASRNKRPTFLKIKKPLSYRKPMDTDLVYIEKSPNYCEEDPVTGSVGTQGRACNKTAPQASGCDLMCCGRGYNTHQYARVWQCNCKFHWCCYVKCNTCSERTEMYTCK

SEQ ID NO: 109 - protein, 318 aa, synthetic construct
  SOURCE 1..318
  REGION 1..318: NOTE = human Wnt7a variant P25A
LGASIICNKIPGLAPRQRAICQSRADAIIVIGEGSQMGLDECQFQFRNGRWNCSALGERTVFGKELKVGSREAAFTYAIIAAGVAHAITAACTQGNLSDCGCDKEKQGQYHRDEGWKWGGCSADIRYGIGFAKVFVDAREIKQNARTLMNLHNNEAGRKILEENMKLECKCHGVSGSCTTKTCWTTLPQFRELGYVLKDKYNEAVHVEPVRASRNKRPTFLKIKKPLSYRKPMDTDLVYIEKSPNYCEEDPVTGSVGTQGRACNKTAPQASGCDLMCCGRGYNTHQYARVWQCNCKFHWCCYVKCNTCSERTEMYTCK

SEQ ID NO: 110 - protein, 318 aa, synthetic construct
  SOURCE 1..318
  REGION 1..318: NOTE = human Wnt7a variant M37A
LGASIICNKIPGLAPRQRAICQSRPDAIIVIGEGSQAGLDECQFQFRNGRWNCSALGERTVFGKELKVGSREAAFTYAIIAAGVAHAITAACTQGNLSDCGCDKEKQGQYHRDEGWKWGGCSADIRYGIGFAKVFVDAREIKQNARTLMNLHNNEAGRKILEENMKLECKCHGVSGSCTTKTCWTTLPQFRELGYVLKDKYNEAVHVEPVRASRNKRPTFLKIKKPLSYRKPMDTDLVYIEKSPNYCEEDPVTGSVGTQGRACNKTAPQASGCDLMCCGRGYNTHQYARVWQCNCKFHWCCYVKCNTCSERTEMYTCK

SEQ ID NO: 111 - protein, 318 aa, synthetic construct
  SOURCE 1..318
  REGION 1..318: NOTE = human Wnt7a variant L39A
LGASIICNKIPGLAPRQRAICQSRPDAIIVIGEGSQMGADECQFQFRNGRWNCSALGERTVFGKELKVGSREAAFTYAIIAAGVAHAITAACTQGNLSDCGCDKEKQGQYHRDEGWKWGGCSADIRYGIGFAKVFVDAREIKQNARTLMNLHNNEAGRKILEENMKLECKCHGVSGSCTTKTCWTTLPQFRELGYVLKDKYNEAVHVEPVRASRNKRPTFLKIKKPLSYRKPMDTDLVYIEKSPNYCEEDPVTGSVGTQGRACNKTAPQASGCDLMCCGRGYNTHQYARVWQCNCKFHWCCYVKCNTCSERTEMYTCK

SEQ ID NO: 112 - protein, 318 aa, synthetic construct
  SOURCE 1..318
  REGION 1..318: NOTE = human Wnt7a variant I28A
LGASIICNKIPGLAPRQRAICQSRPDAAIVIGEGSQMGLDECQFQFRNGRWNCSALGERTVFGKELKVGSREAAFTYAIIAAGVAHAITAACTQGNLSDCGCDKEKQGQYHRDEGWKWGGCSADIRYGIGFAKVFVDAREIKQNARTLMNLHNNEAGRKILEENMKLECKCHGVSGSCTTKTCWTTLPQFRELGYVLKDKYNEAVHVEPVRASRNKRPTFLKIKKPLSYRKPMDTDLVYIEKSPNYCEEDPVTGSVGTQGRACNKTAPQASGCDLMCCGRGYNTHQYARVWQCNCKFHWCCYVKCNTCSERTEMYTCK

SEQ ID NO: 113 - protein, 318 aa, synthetic construct
  SOURCE 1..318
  REGION 1..318: NOTE = human Wnt7a variant R50A
LGASIICNKIPGLAPRQRAICQSRPDAIIVIGEGSQMGLDECQFQFRNGAWNCSALGERTVFGKELKVGSREAAFTYAIIAAGVAHAITAACTQGNLSDCGCDKEKQGQYHRDEGWKWGGCSADIRYGIGFAKVFVDAREIKQNARTLMNLHNNEAGRKILEENMKLECKCHGVSGSCTTKTCWTTLPQFRELGYVLKDKYNEAVHVEPVRASRNKRPTFLKIKKPLSYRKPMDTDLVYIEKSPNYCEEDPVTGSVGTQGRACNKTAPQASGCDLMCCGRGYNTHQYARVWQCNCKFHWCCYVKCNTCSERTEMYTCK

SEQ ID NO: 114 - protein, 318 aa, synthetic construct
  SOURCE 1..318
  REGION 1..318: NOTE = human Wnt7a variant V68A
LGASIICNKIPGLAPRQRAICQSRPDAIIVIGEGSQMGLDECQFQFRNGRWNCSALGERTVFGKELKAGSREAAFTYAIIAAGVAHAITAACTQGNLSDCGCDKEKQGQYHRDEGWKWGGCSADIRYGIGFAKVFVDAREIKQNARTLMNLHNNEAGRKILEENMKLECKCHGVSGSCTTKTCWTTLPQFRELGYVLKDKYNEAVHVEPVRASRNKRPTFLKIKKPLSYRKPMDTDLVYIEKSPNYCEEDPVTGSVGTQGRACNKTAPQASGCDLMCCGRGYNTHQYARVWQCNCKFHWCCYVKCNTCSERTEMYTCK

SEQ ID NO: 115 - protein, 318 aa, synthetic construct
  SOURCE 1..318
  REGION 1..318: NOTE = human Wnt7a variant F135A
LGASIICNKIPGLAPRQRAICQSRPDAIIVIGEGSQMGLDECQFQFRNGRWNCSALGERTVFGKELKVGSREAAFTYAIIAAGVAHAITAACTQGNLSDCGCDKEKQGQYHRDEGWKWGGCSADIRYGIGFAKVAVDAREIKQNARTLMNLHNNEAGRKILEENMKLECKCHGVSGSCTTKTCWTTLPQFRELGYVLKDKYNEAVHVEPVRASRNKRPTFLKIKKPLSYRKPMDTDLVYIEKSPNYCEEDPVTGSVGTQGRACNKTAPQASGCDLMCCGRGYNTHQYARVWQCNCKFHWCCYVKCNTCSERTEMYTCK

SEQ ID NO: 116 - protein, 318 aa, synthetic construct
  SOURCE 1..318
  REGION 1..318: NOTE = human Wnt7a variant R146A
LGASIICNKIPGLAPRQRAICQSRPDAIIVIGEGSQMGLDECQFQFRNGRWNCSALGERTVFGKELKVGSREAAFTYAIIAAGVAHAITAACTQGNLSDCGCDKEKQGQYHRDEGWKWGGCSADIRYGIGFAKVFVDAREIKQNAATLMNLHNNEAGRKILEENMKLECKCHGVSGSCTTKTCWTTLPQFRELGYVLKDKYNEAVHVEPVRASRNKRPTFLKIKKPLSYRKPMDTDLVYIEKSPNYCEEDPVTGSVGTQGRACNKTAPQASGCDLMCCGRGYNTHQYARVWQCNCKFHWCCYVKCNTCSERTEMYTCK

SEQ ID NO: 117 - protein, 318 aa, synthetic construct
  SOURCE 1..318
  REGION 1..318: NOTE = human Wnt7a variant K159S
LGASIICNKIPGLAPRQRAICQSRPDAIIVIGEGSQMGLDECQFQFRNGRWNCSALGERTVFGKELKVGSREAAFTYAIIAAGVAHAITAACTQGNLSDCGCDKEKQGQYHRDEGWKWGGCSADIRYGIGFAKVFVDAREIKQNARTLMNLHNNEAGRSILEENMKLECKCHGVSGSCTTKTCWTTLPQFRELGYVLKDKYNEAVHVEPVRASRNKRPTFLKIKKPLSYRKPMDTDLVYIEKSPNYCEEDPVTGSVGTQGRACNKTAPQASGCDLMCCGRGYNTHQYARVWQCNCKFHWCCYVKCNTCSERTEMYTCK

SEQ ID NO: 118 - protein, 318 aa, synthetic construct
  SOURCE 1..318
  REGION 1..318: NOTE = human Wnt7a variant K159L
LGASIICNKIPGLAPRQRAICQSRPDAIIVIGEGSQMGLDECQFQFRNGRWNCSALGERTVFGKELKVGSREAAFTYAIIAAGVAHAITAACTQGNLSDCGCDKEKQGQYHRDEGWKWGGCSADIRYGIGFAKVFVDAREIKQNARTLMNLHNNEAGRLILEENMKLECKCHGVSGSCTTKTCWTTLPQFRELGYVLKDKYNEAVHVEPVRASRNKRPTFLKIKKPLSYRKPMDTDLVYIEKSPNYCEEDPVTGSVGTQGRACNKTAPQASGCDLMCCGRGYNTHQYARVWQCNCKFHWCCYVKCNTCSERTEMYTCK

SEQ ID NO: 119 - protein, 318 aa, synthetic construct
  SOURCE 1..318
  REGION 1..318: NOTE = human Wnt7a variant K200A
LGASIICNKIPGLAPRQRAICQSRPDAIIVIGEGSQMGLDECQFQFRNGRWNCSALGERTVFGKELKVGSREAAFTYAIIAAGVAHAITAACTQGNLSDCGCDKEKQGQYHRDEGWKWGGCSADIRYGIGFAKVFVDAREIKQNARTLMNLHNNEAGRKILEENMKLECKCHGVSGSCTTKTCWTTLPQFRELGYVLKDAYNEAVHVEPVRASRNKRPTFLKIKKPLSYRKPMDTDLVYIEKSPNYCEEDPVTGSVGTQGRACNKTAPQASGCDLMCCGRGYNTHQYARVWQCNCKFHWCCYVKCNTCSERTEMYTCK

SEQ ID NO: 120 - protein, 318 aa, synthetic construct
  SOURCE 1..318
  REGION 1..318: NOTE = human Wnt7a variant R214A
LGASIICNKIPGLAPRQRAICQSRPDAIIVIGEGSQMGLDECQFQFRNGRWNCSALGERTVFGKELKVGSREAAFTYAIIAAGVAHAITAACTQGNLSDCGCDKEKQGQYHRDEGWKWGGCSADIRYGIGFAKVFVDAREIKQNARTLMNLHNNEAGRKILEENMKLECKCHGVSGSCTTKTCWTTLPQFRELGYVLKDKYNEAVHVEPVRASANKRPTFLKIKKPLSYRKPMDTDLVYIEKSPNYCEEDPVTGSVGTQGRACNKTAPQASGCDLMCCGRGYNTHQYARVWQCNCKFHWCCYVKCNTCSERTEMYTCK

SEQ ID NO: 121 - protein, 318 aa, synthetic construct; identical to SEQ ID NO: 51
  REGION 1..318: NOTE = human Wnt7a variant P218A
  SOURCE 1..318